European Patent Application EP 4 516 909 A1, published March 5, 2025. Title: 靶向CD19的嵌合抗原受体及其应用. Applicant: 上海先博生物科技有限公司. The sequence listing filed with the application follows.

SEQUENCE LISTING (57 sequences)

SEQ ID NO: 1 - protein, 119 aa, synthetic construct
QVQLQQPGAELVVPGTSVKLSCKASGYTFTNYWMHWVKQRPGQGLEWIGEIDPSDNYANYNQEFQGKATLTVDKSSSTAYMQLSSLTSDDSAVYYCARHDGYFGALDYWGQGTSVTVSS

SEQ ID NO: 2 - protein, 110 aa, synthetic construct
EIVLTQSPTTMAASPGEKITITCSASSSISSNYLHWYQQKPGFSPKFLIYRTSNLASGVPARFSGSGSGTSYSLTIGTMEAEDVATYYCQQASSIPRMFTFGSGTKLEIK

SEQ ID NO: 3 - protein, 120 aa, synthetic construct
EVQLQQSGPELVKPGASVKMSCKASGYTFTDYVMHWVRQTPGQGLEWIGYFNPYNDGTNYNEKFKVKATLTSDKSSTTAYMELSSLTSEDSAVYYCARGVYYYGRDFDYWGQGTTLTVSS

SEQ ID NO: 4 - protein, 112 aa, synthetic construct
DVVLTQTPLSLPVSLGDQASISCRSSQSLENSNGNSYLNWYLQKPGQSPQLLIYRVSNRFSGVLDRFSGSGSGTDFTLKISRVEAEDLGVYFCLQITHVPWTFGGGTKLEIK

SEQ ID NO: 5 - protein, 114 aa, synthetic construct
QVQLQQSGAELVRPGASVTLSCKASGYTFPDYEIHWVKQTPVHGLEWIGAIDPETGGIGYNQKFTGKAMLTADKSSSTAYMELRSLTSEDSAVYFCTRNYGSRWGQGSTLTVSS

SEQ ID NO: 6 - protein, 112 aa, synthetic construct
DVVMTQTPLTLSVTIGQSASISCKSSQSLLESDGKTYLNWLLQRPGQSPKRLIYLVSKLDSGVPDRFTGSASGTDFTLKISRVEAEDLGVYYCWQGTHFPWTFGGGTKLEIK

SEQ ID NO: 7 - protein, 120 aa, synthetic construct
EVKLQESGPGLVAPSQSLSVTCTVSGVSLPDYGVSWIRQPPRKGLEWLGVIWGSETTYYNSALKSRLTIIKDNSKSQVFLKMNSLQTDDTAIYYCAKHYYYGGSYAMDYWGQGTSVTVSS

SEQ ID NO: 8 - protein, 107 aa, synthetic construct
DIQMTQTTSSLSASLGDRVTISCRASQDISKYLNWYQQKPDGTVKLLIYHTSRLHSGVPSRFSGSGSGTDYSLTISNLEQEDIATYFCQQGNTLPYTFGGGTKLEIT

SEQ ID NO: 9 - protein, 5 aa, synthetic construct
NYWMH

SEQ ID NO: 10 - protein, 17 aa, synthetic construct
EIDPSDNYANYNQEFQG

SEQ ID NO: 11 - protein, 10 aa, synthetic construct
HDGYFGALDY

SEQ ID NO: 12 - protein, 12 aa, synthetic construct
SASSSISSNYLH

SEQ ID NO: 13 - protein, 7 aa, synthetic construct
RTSNLAS

SEQ ID NO: 14 - protein, 11 aa, synthetic construct
QQASSIPRMFT

SEQ ID NO: 15 - protein, 5 aa, synthetic construct
DYVMH

SEQ ID NO: 16 - protein, 17 aa, synthetic construct
YFNPYNDGTNYNEKFKV

SEQ ID NO: 17 - protein, 11 aa, synthetic construct
GVYYYGRDFDY

SEQ ID NO: 18 - protein, 16 aa, synthetic construct
RSSQSLENSNGNSYLN

SEQ ID NO: 19 - protein, 7 aa, synthetic construct
RVSNRFS

SEQ ID NO: 20 - protein, 9 aa, synthetic construct
LQITHVPWT

SEQ ID NO: 21 - protein, 5 aa, synthetic construct
DYEIH

SEQ ID NO: 22 - protein, 17 aa, synthetic construct
AIDPETGGIGYNQKFTG

SEQ ID NO: 23 - protein, 5 aa, synthetic construct
NYGSR

SEQ ID NO: 24 - protein, 16 aa, synthetic construct
KSSQSLLESDGKTYLN

SEQ ID NO: 25 - protein, 7 aa, synthetic construct
LVSKLDS

SEQ ID NO: 26 - protein, 9 aa, synthetic construct
WQGTHFPWT

SEQ ID NO: 27 - protein, 5 aa, synthetic construct
DYGVS

SEQ ID NO: 28 - protein, 16 aa, synthetic construct
VIWGSETTYYNSALKS

SEQ ID NO: 29 - protein, 12 aa, synthetic construct
HYYYGGSYAMDY

SEQ ID NO: 30 - protein, 11 aa, synthetic construct
RASQDISKYLN

SEQ ID NO: 31 - protein, 7 aa, synthetic construct
HTSRLHS

SEQ ID NO: 32 - protein, 9 aa, synthetic construct
QQGNTLPYT

SEQ ID NO: 33 - protein, 21 aa, synthetic construct
MALPVTALLLPLALLLHAARP

SEQ ID NO: 34 - protein, 688 aa, synthetic construct
MALPVTALLLPLALLLHAARPLEEIVLTQSPTTMAASPGEKITITCSASSSISSNYLHWYQQKPGFSPKFLIYRTSNLASGVPARFSGSGSGTSYSLTIGTMEAEDVATYYCQQASSIPRMFTFGSGTKLEIKGSTSGSGKPGSGEGSTKGQVQLQQPGAELVVPGTSVKLSCKASGYTFTNYWMHWVKQRPGQGLEWIGEIDPSDNYANYNQEFQGKATLTVDKSSSTAYMQLSSLTSDDSAVYYCARHDGYFGALDYWGQGTSVTVSSGSFVPVFLPAKRTTTPAPRPPTPAPTIASQPLSLRPEACRPAAGGAVHTRGLDFACDIYIWAPLAGTCGVLLLSLVITLYCRSKRSRLLHSDYMNMTPRRPGPTRKHYQPYAPPRDFAAYRSRVKFSRSADAPAYQQGQNQLYNELNLGRREEYDVLDKRRGRDPEMGGKPRRKNPQEGLYNELQKDKMAEAYSEIGMKGERRRGKGHDGLYQGLSTATKDTYDALHMQALPPRGSGATNFSLLKQAGDVEENPGPMRISKPHLRSISIQCYLCLLLNSHFLTEAGIHVFILGCFSAGLPKTEANWVNVISDLKKIEDLIQSMHIDATLYTESDVHPSCKVTAMKCFLLELQVISLESGDASIHDTVENLIILANNSLSSNGNVTESGCKECEELEEKNIKEFLQSFVHIVQMFINTS

SEQ ID NO: 35 - protein, 691 aa, synthetic construct
MALPVTALLLPLALLLHAARPLEDVVLTQTPLSLPVSLGDQASISCRSSQSLENSNGNSYLNWYLQKPGQSPQLLIYRVSNRFSGVLDRFSGSGSGTDFTLKISRVEAEDLGVYFCLQITHVPWTFGGGTKLEIKGSTSGSGKPGSGEGSTKGEVQLQQSGPELVKPGASVKMSCKASGYTFTDYVMHWVRQTPGQGLEWIGYFNPYNDGTNYNEKFKVKATLTSDKSSTTAYMELSSLTSEDSAVYYCARGVYYYGRDFDYWGQGTTLTVSSGSFVPVFLPAKRTTTPAPRPPTPAPTIASQPLSLRPEACRPAAGGAVHTRGLDFACDIYIWAPLAGTCGVLLLSLVITLYCRSKRSRLLHSDYMNMTPRRPGPTRKHYQPYAPPRDFAAYRSRVKFSRSADAPAYQQGQNQLYNELNLGRREEYDVLDKRRGRDPEMGGKPRRKNPQEGLYNELQKDKMAEAYSEIGMKGERRRGKGHDGLYQGLSTATKDTYDALHMQALPPRGSGATNFSLLKQAGDVEENPGPMRISKPHLRSISIQCYLCLLLNSHFLTEAGIHVFILGCFSAGLPKTEANWVNVISDLKKIEDLIQSMHIDATLYTESDVHPSCKVTAMKCFLLELQVISLESGDASIHDTVENLIILANNSLSSNGNVTESGCKECEELEEKNIKEFLQSFVHIVQMFINTS

SEQ ID NO: 36 - protein, 685 aa, synthetic construct
MALPVTALLLPLALLLHAARPLEDVVMTQTPLTLSVTIGQSASISCKSSQSLLESDGKTYLNWLLQRPGQSPKRLIYLVSKLDSGVPDRFTGSASGTDFTLKISRVEAEDLGVYYCWQGTHFPWTFGGGTKLEIKGSTSGSGKPGSGEGSTKGQVQLQQSGAELVRPGASVTLSCKASGYTFPDYEIHWVKQTPVHGLEWIGAIDPETGGIGYNQKFTGKAMLTADKSSSTAYMELRSLTSEDSAVYFCTRNYGSRWGQGSTLTVSSGSFVPVFLPAKRTTTPAPRPPTPAPTIASQPLSLRPEACRPAAGGAVHTRGLDFACDIYIWAPLAGTCGVLLLSLVITLYCRSKRSRLLHSDYMNMTPRRPGPTRKHYQPYAPPRDFAAYRSRVKFSRSADAPAYQQGQNQLYNELNLGRREEYDVLDKRRGRDPEMGGKPRRKNPQEGLYNELQKDKMAEAYSEIGMKGERRRGKGHDGLYQGLSTATKDTYDALHMQALPPRGSGATNFSLLKQAGDVEENPGPMRISKPHLRSISIQCYLCLLLNSHFLTEAGIHVFILGCFSAGLPKTEANWVNVISDLKKIEDLIQSMHIDATLYTESDVHPSCKVTAMKCFLLELQVISLESGDASIHDTVENLIILANNSLSSNGNVTESGCKECEELEEKNIKEFLQSFVHIVQMFINTS

SEQ ID NO: 37 - protein, 686 aa, synthetic construct
MALPVTALLLPLALLLHAARPLEDIQMTQTTSSLSASLGDRVTISCRASQDISKYLNWYQQKPDGTVKLLIYHTSRLHSGVPSRFSGSGSGTDYSLTISNLEQEDIATYFCQQGNTLPYTFGGGTKLEITGSTSGSGKPGSGEGSTKGEVKLQESGPGLVAPSQSLSVTCTVSGVSLPDYGVSWIRQPPRKGLEWLGVIWGSETTYYNSALKSRLTIIKDNSKSQVFLKMNSLQTDDTAIYYCAKHYYYGGSYAMDYWGQGTSVTVSSGSFVPVFLPAKRTTTPAPRPPTPAPTIASQPLSLRPEACRPAAGGAVHTRGLDFACDIYIWAPLAGTCGVLLLSLVITLYCRSKRSRLLHSDYMNMTPRRPGPTRKHYQPYAPPRDFAAYRSRVKFSRSADAPAYQQGQNQLYNELNLGRREEYDVLDKRRGRDPEMGGKPRRKNPQEGLYNELQKDKMAEAYSEIGMKGERRRGKGHDGLYQGLSTATKDTYDALHMQALPPRGSGATNFSLLKQAGDVEENPGPMRISKPHLRSISIQCYLCLLLNSHFLTEAGIHVFILGCFSAGLPKTEANWVNVISDLKKIEDLIQSMHIDATLYTESDVHPSCKVTAMKCFLLELQVISLESGDASIHDTVENLIILANNSLSSNGNVTESGCKECEELEEKNIKEFLQSFVHIVQMFINTS

SEQ ID NO: 38 - protein, 110 aa, synthetic construct
EIVLTQSPATLSLSPGERATLSCSASSSISSNYLHWYQQKPGQAPRFLIYRTSNLASGIPARFSGSGSGTDFTLTISSLEPEDFAVYYCQQASSIPRMFTFGQGTKLEIK

SEQ ID NO: 39 - protein, 110 aa, synthetic construct
EIVLTQSPDFQSVTPKEKVTITCSASSSISSNYLHWYQQKPDQSPKFLIYRTSNLASGVPSRFSGSGSGTDFTLTINSLEAEDAATYYCQQASSIPRMFTFGQGTKLEIK

SEQ ID NO: 40 - protein, 119 aa, synthetic construct
EVQLVQSGAEVKKPGASVKVSCKASGYTFTNYWMHWVRQRPGQGLEWMGEIDPSDNYANYNQEFQGRVTITVDKSASTAYMELSSLRSEDTAVYYCARHDGYFGALDYWGQGTTVTVSS

SEQ ID NO: 41 - protein, 119 aa, synthetic construct
EVQLQQSGAEVKKPGASVKVSCKASGYTFTNYWMHWVRQRPGQGLEWMGEIDPSDNYANYNQEFQGRVTITVDKSASTAYMELSSLRSEDTAVYYCARHDGYFGALDYWGQGTTVTVSS

SEQ ID NO: 42 - protein, 107 aa, synthetic construct
DIQMTQSPSSLSASVGDRVTITCRASQDISKYLNWYQQKPGGAVKLLIYHTSRLHSGVPSRFSGSGSGTDYTLTISSLQPEDFATYYCQQGNTLPYTFGGGTKVEIK

SEQ ID NO: 43 - protein, 120 aa, synthetic construct
EVTLKESGPVLVKPTETLTLTCTVSGFSLSDYGVSWIRQPPGKALEWLAVIWGSETTYYNSALKSRLTISKDTSKSQVVLTMTNMDPVDTATYYCAKHYYYGGSYAMDYWGQGTTVTVSS

SEQ ID NO: 44 - protein, 688 aa, synthetic construct
MALPVTALLLPLALLLHAARPLEEIVLTQSPATLSLSPGERATLSCSASSSISSNYLHWYQQKPGQAPRFLIYRTSNLASGIPARFSGSGSGTDFTLTISSLEPEDFAVYYCQQASSIPRMFTFGQGTKLEIKGSTSGSGKPGSGEGSTKGEVQLQQSGAEVKKPGASVKVSCKASGYTFTNYWMHWVRQRPGQGLEWMGEIDPSDNYANYNQEFQGRVTITVDKSASTAYMELSSLRSEDTAVYYCARHDGYFGALDYWGQGTTVTVSSGSFVPVFLPAKRTTTPAPRPPTPAPTIASQPLSLRPEACRPAAGGAVHTRGLDFACDIYIWAPLAGTCGVLLLSLVITLYCRSKRSRLLHSDYMNMTPRRPGPTRKHYQPYAPPRDFAAYRSRVKFSRSADAPAYQQGQNQLYNELNLGRREEYDVLDKRRGRDPEMGGKPRRKNPQEGLYNELQKDKMAEAYSEIGMKGERRRGKGHDGLYQGLSTATKDTYDALHMQALPPRGSGATNFSLLKQAGDVEENPGPMRISKPHLRSISIQCYLCLLLNSHFLTEAGIHVFILGCFSAGLPKTEANWVNVISDLKKIEDLIQSMHIDATLYTESDVHPSCKVTAMKCFLLELQVISLESGDASIHDTVENLIILANNSLSSNGNVTESGCKECEELEEKNIKEFLQSFVHIVQMFINTS

SEQ ID NO: 45 - protein, 688 aa, synthetic construct
MALPVTALLLPLALLLHAARPLEEIVLTQSPDFQSVTPKEKVTITCSASSSISSNYLHWYQQKPDQSPKFLIYRTSNLASGVPSRFSGSGSGTDFTLTINSLEAEDAATYYCQQASSIPRMFTFGQGTKLEIKGSTSGSGKPGSGEGSTKGEVQLVQSGAEVKKPGASVKVSCKASGYTFTNYWMHWVRQRPGQGLEWMGEIDPSDNYANYNQEFQGRVTITVDKSASTAYMELSSLRSEDTAVYYCARHDGYFGALDYWGQGTTVTVSSGSFVPVFLPAKRTTTPAPRPPTPAPTIASQPLSLRPEACRPAAGGAVHTRGLDFACDIYIWAPLAGTCGVLLLSLVITLYCRSKRSRLLHSDYMNMTPRRPGPTRKHYQPYAPPRDFAAYRSRVKFSRSADAPAYQQGQNQLYNELNLGRREEYDVLDKRRGRDPEMGGKPRRKNPQEGLYNELQKDKMAEAYSEIGMKGERRRGKGHDGLYQGLSTATKDTYDALHMQALPPRGSGATNFSLLKQAGDVEENPGPMRISKPHLRSISIQCYLCLLLNSHFLTEAGIHVFILGCFSAGLPKTEANWVNVISDLKKIEDLIQSMHIDATLYTESDVHPSCKVTAMKCFLLELQVISLESGDASIHDTVENLIILANNSLSSNGNVTESGCKECEELEEKNIKEFLQSFVHIVQMFINTS

SEQ ID NO: 46 - protein, 686 aa, synthetic construct
MALPVTALLLPLALLLHAARPLEDIQMTQSPSSLSASVGDRVTITCRASQDISKYLNWYQQKPGGAVKLLIYHTSRLHSGVPSRFSGSGSGTDYTLTISSLQPEDFATYYCQQGNTLPYTFGGGTKVEIKGSTSGSGKPGSGEGSTKGEVTLKESGPVLVKPTETLTLTCTVSGFSLSDYGVSWIRQPPGKALEWLAVIWGSETTYYNSALKSRLTISKDTSKSQVVLTMTNMDPVDTATYYCAKHYYYGGSYAMDYWGQGTTVTVSSGSFVPVFLPAKRTTTPAPRPPTPAPTIASQPLSLRPEACRPAAGGAVHTRGLDFACDIYIWAPLAGTCGVLLLSLVITLYCRSKRSRLLHSDYMNMTPRRPGPTRKHYQPYAPPRDFAAYRSRVKFSRSADAPAYQQGQNQLYNELNLGRREEYDVLDKRRGRDPEMGGKPRRKNPQEGLYNELQKDKMAEAYSEIGMKGERRRGKGHDGLYQGLSTATKDTYDALHMQALPPRGSGATNFSLLKQAGDVEENPGPMRISKPHLRSISIQCYLCLLLNSHFLTEAGIHVFILGCFSAGLPKTEANWVNVISDLKKIEDLIQSMHIDATLYTESDVHPSCKVTAMKCFLLELQVISLESGDASIHDTVENLIILANNSLSSNGNVTESGCKECEELEEKNIKEFLQSFVHIVQMFINTS

SEQ ID NO: 47 - protein, 55 aa, synthetic construct
FVPVFLPAKRTTTPAPRPPTPAPTIASQPLSLRPEACRPAAGGAVHTRGLDFACD

SEQ ID NO: 48 - protein, 24 aa, synthetic construct
IYIWAPLAGTCGVLLLSLVITLYC

SEQ ID NO: 49 - protein, 112 aa, synthetic construct
RVKFSRSADAPAYQQGQNQLYNELNLGRREEYDVLDKRRGRDPEMGGKPRRKNPQEGLYNELQKDKMAEAYSEIGMKGERRRGKGHDGLYQGLSTATKDTYDALHMQALPPR

SEQ ID NO: 50 - protein, 41 aa, synthetic construct
RSKRSRLLHSDYMNMTPRRPGPTRKHYQPYAPPRDFAAYRS

SEQ ID NO: 51 - protein, 247 aa, synthetic construct
EIVLTQSPTTMAASPGEKITITCSASSSISSNYLHWYQQKPGFSPKFLIYRTSNLASGVPARFSGSGSGTSYSLTIGTMEAEDVATYYCQQASSIPRMFTFGSGTKLEIKGSTSGSGKPGSGEGSTKGQVQLQQPGAELVVPGTSVKLSCKASGYTFTNYWMHWVKQRPGQGLEWIGEIDPSDNYANYNQEFQGKATLTVDKSSSTAYMQLSSLTSDDSAVYYCARHDGYFGALDYWGQGTSVTVSS

SEQ ID NO: 52 - protein, 250 aa, synthetic construct
DVVLTQTPLSLPVSLGDQASISCRSSQSLENSNGNSYLNWYLQKPGQSPQLLIYRVSNRFSGVLDRFSGSGSGTDFTLKISRVEAEDLGVYFCLQITHVPWTFGGGTKLEIKGSTSGSGKPGSGEGSTKGEVQLQQSGPELVKPGASVKMSCKASGYTFTDYVMHWVRQTPGQGLEWIGYFNPYNDGTNYNEKFKVKATLTSDKSSTTAYMELSSLTSEDSAVYYCARGVYYYGRDFDYWGQGTTLTVSS

SEQ ID NO: 53 - protein, 244 aa, synthetic construct
DVVMTQTPLTLSVTIGQSASISCKSSQSLLESDGKTYLNWLLQRPGQSPKRLIYLVSKLDSGVPDRFTGSASGTDFTLKISRVEAEDLGVYYCWQGTHFPWTFGGGTKLEIKGSTSGSGKPGSGEGSTKGQVQLQQSGAELVRPGASVTLSCKASGYTFPDYEIHWVKQTPVHGLEWIGAIDPETGGIGYNQKFTGKAMLTADKSSSTAYMELRSLTSEDSAVYFCTRNYGSRWGQGSTLTVSS

SEQ ID NO: 54 - protein, 245 aa, synthetic construct
DIQMTQTTSSLSASLGDRVTISCRASQDISKYLNWYQQKPDGTVKLLIYHTSRLHSGVPSRFSGSGSGTDYSLTISNLEQEDIATYFCQQGNTLPYTFGGGTKLEITGSTSGSGKPGSGEGSTKGEVKLQESGPGLVAPSQSLSVTCTVSGVSLPDYGVSWIRQPPRKGLEWLGVIWGSETTYYNSALKSRLTIIKDNSKSQVFLKMNSLQTDDTAIYYCAKHYYYGGSYAMDYWGQGTSVTVSS

SEQ ID NO: 55 - protein, 247 aa, synthetic construct
EIVLTQSPATLSLSPGERATLSCSASSSISSNYLHWYQQKPGQAPRFLIYRTSNLASGIPARFSGSGSGTDFTLTISSLEPEDFAVYYCQQASSIPRMFTFGQGTKLEIKGSTSGSGKPGSGEGSTKGEVQLQQSGAEVKKPGASVKVSCKASGYTFTNYWMHWVRQRPGQGLEWMGEIDPSDNYANYNQEFQGRVTITVDKSASTAYMELSSLRSEDTAVYYCARHDGYFGALDYWGQGTTVTVSS

SEQ ID NO: 56 - protein, 247 aa, synthetic construct
EIVLTQSPDFQSVTPKEKVTITCSASSSISSNYLHWYQQKPDQSPKFLIYRTSNLASGVPSRFSGSGSGTDFTLTINSLEAEDAATYYCQQASSIPRMFTFGQGTKLEIKGSTSGSGKPGSGEGSTKGEVQLVQSGAEVKKPGASVKVSCKASGYTFTNYWMHWVRQRPGQGLEWMGEIDPSDNYANYNQEFQGRVTITVDKSASTAYMELSSLRSEDTAVYYCARHDGYFGALDYWGQGTTVTVSS

SEQ ID NO: 57 - protein, 245 aa, synthetic construct
DIQMTQSPSSLSASVGDRVTITCRASQDISKYLNWYQQKPGGAVKLLIYHTSRLHSGVPSRFSGSGSGTDYTLTISSLQPEDFATYYCQQGNTLPYTFGGGTKVEIKGSTSGSGKPGSGEGSTKGEVTLKESGPVLVKPTETLTLTCTVSGFSLSDYGVSWIRQPPGKALEWLAVIWGSETTYYNSALKSRLTISKDTSKSQVVLTMTNMDPVDTATYYCAKHYYYGGSYAMDYWGQGTTVTVSS